European Patent Application EP 4 458 861 A1, published November 6, 2024. Title: CD3-TARGETING ANTIBODY AND MULTISPECIFIC ANTIBODY AND USE THEREOF. Applicant: SICHUAN HUIYU PHARMACEUTICAL CO., LTD. The sequence listing filed with the application follows.

SEQUENCE LISTING (176 sequences)

SEQ ID NO: 1 - protein, 125 aa, synthetic construct
  source 1..125: note = CD3 antibody VH-1
EVQLVESGGGLVQPGGSLRLSCAASGFTFNTYAMNWVRQAPGKGLEWVARIRSKYNNYATYYADSVKGRFTISRDDSKSILYLQMNNLKTEDTAMYYCVRHANFLNSYVSWFAYWGQGTLVTVSS

SEQ ID NO: 2 - protein, 125 aa, synthetic construct
  source 1..125: note = CD3 antibody VH-2
EVQLVESGGGLVQPGGSLRLSCAASGFTFNTYAMNWVRQAPGKGLEWVARIRSKYNNYATYYADSVKGRFTISRDDSKSSLYLQMNSLKTEDTAMYYCVRAKNFGNSYVSWFAYWGQGTLVTVSS

SEQ ID NO: 3 - protein, 125 aa, synthetic construct
  source 1..125: note = CD3 antibody VH-3
EVQLVESGGGLVQPGGSLRLSCAASGFTFNTYAMNWVRQAPGKGLEWVARIRSKYNNYATYYADSVKDRFTISRDDSKSILYLQMNSLKTEDTAMYYCVRHGNFGNSYVSWFEYWGQGTLVTVSS

SEQ ID NO: 4 - protein, 125 aa, synthetic construct
  source 1..125: note = CD3 antibody VH-4
EVQLVESGGGLVQPGGSLRLSCAASGFTFNTYAMNWVRQAPGKGLEWVARIRSKYNNYATYYADSVKDRFTISRDDSKSILYLQMNNLKTEDTAVYYCVRHGNFQNSYVSWFQYWGQGTLVTVSS

SEQ ID NO: 5 - protein, 125 aa, synthetic construct
  source 1..125: note = CD3 antibody VH-5
EVQLVESGGGLVQPGGSLRLSCAASGFTFNTYAMNWVRQAPGKGLEWVARIRSKYNNYATYYADSVKDRFTISRDDSKSILYLQMNSLKTEDTAVYYCVRHGNFKNSYVSWFAYWGQGTLVTVSS

SEQ ID NO: 6 - protein, 125 aa, synthetic construct
  source 1..125: note = CD3 antibody VH-6
EVQLVESGGGLVQPGGSLRLSCAASGFTFNTYAMNWVRQAPGKGLEWVARIRSKYNNYATYYADSVKGRFTISRDDSKSSLYLQMNSLKTEDTAMYYCVRHGNFYNSYVSWFAHWGQGTLVTVSS

SEQ ID NO: 7 - protein, 125 aa, synthetic construct
  source 1..125: note = CD3 antibody VH-7
EVQLVESGGGLVQPGGSLRLSCAASGFTFNTYAMNWVRQAPGKGLEWVARIRSKYNNYATYYADSVKDRFTISRDDSKSSLYLQMNNLKTEDTAMYYCVRAGNFGNSYVSWFEYWGQGTLVTVSS

SEQ ID NO: 8 - protein, 125 aa, synthetic construct
  source 1..125: note = CD3 antibody VH-8
EVQLVESGGGLVQPGGSLRLSCAASGFTFNTYAMNWVRQAPGKGLEWVARIRSKYNNYATYYADSVKDRFTISRDDSKSSLYLQMNNLKTEDTAMYYCVRHGNFGNTYVSWFAMWGQGTLVTVSS

SEQ ID NO: 9 - protein, 125 aa, synthetic construct
  source 1..125: note = CD3 antibody VH-9
EVQLVESGGGLVQPGGSLRLSCAASGFTFNTYAMNWVRQAPGKGLEWVARIRSKYNNYATYYADSVKGRFTISRDDSKSILYLQMNSLKTEDTAMYYCVRHGNFGNSYVSWFKYWGQGTLVTVSS

SEQ ID NO: 10 - protein, 125 aa, synthetic construct
  source 1..125: note = CD3 antibody VH-10
EVQLVESGGGLVQPGGSLRLSCAASGFTFNTYAMNWVRQAPGKGLEWVARIRSKYNNYATYYADSVKDRFTISRDDSKSSLYLQMNSLKTEDTAVYYCVRHSNFRNSYVSWFAYWGQGTLVTVSS

SEQ ID NO: 11 - protein, 125 aa, synthetic construct
  source 1..125: note = CD3 antibody VH-11
EVQLVESGGGLVQPGGSLRLSCAASGFTFNTYAMNWVRQAPGKGLEWVARIRSKYNNYATYYADSVKDRFTISRDDSKSSLYLQMNSLKTEDTAVYYCVRHSNFVNSYVSWFAYWGQGTLVTVSS

SEQ ID NO: 12 - protein, 125 aa, synthetic construct
  source 1..125: note = CD3 antibody VH-12
EVQLVESGGGLVQPGGSLRLSCAASGFTFNTYAMNWVRQAPGKGLEWVARIRSKYNNYATYYADSVKGRFTISRDDSKSSLYLQMNNLKTEDTAMYYCVRHSNFPNSYVSWFAYWGQGTLVTVSS

SEQ ID NO: 13 - protein, 125 aa, synthetic construct
  source 1..125: note = CD3 antibody VH-13
EVQLVESGGGLVQPGGSLRLSCAASGFTFNTYAMNWVRQAPGKGLEWVARIRSKYNNYATYYADSVKGRFTISRDDSKSSLYLQMNSLKTEDTAVYYCVRHGNFKNSYGSWFAYWGQGTLVTVSS

SEQ ID NO: 14 - protein, 125 aa, synthetic construct
  source 1..125: note = CD3 antibody VH-14
EVQLVESGGGLVQPGGSLRLSCAASGFTFNTYAMNWVRQAPGKGLEWVARIRSKYNNYATYYADSVKDRFTISRDDSKSSLYLQMNSLKTEDTAMYYCVRHSNFGNSYVSWFEYWGQGTLVTVSS

SEQ ID NO: 15 - protein, 125 aa, synthetic construct
  source 1..125: note = CD3 antibody VH-15
EVQLVESGGGLVQPGGSLRLSCAASGFTFNTYAMNWVRQAPGKGLEWVARIRSKYNNYATYYADSVKDRFTISRDDSKSSLYLQMNSLKTEDTAMYYCVRHGDPGNSYVSWFAYWGQGTLVTVSS

SEQ ID NO: 16 - protein, 125 aa, synthetic construct
  source 1..125: note = CD3 antibody VH-16
EVQLVESGGGLVQPGGSLRLSCAASGFTFNTYAMNWVRQAPGKGLEWVARIRSKYNNYATYYADSVKGRFTISRDDSKSILYLQMNSLKTEDTAVYYCVRHGNFGNSYVSWFQYWGQGTLVTVSS

SEQ ID NO: 17 - protein, 125 aa, synthetic construct
  source 1..125: note = CD3 antibody VH-17
EVQLVESGGGLVQPGGSLRLSCAASGFTFNTYAMNWVRQAPGKGLEWVARIRSKYNNYATYYADSVKDRFTISRDDSKSILYLQMNSLKTEDTAMYYCVRHGNFWNSYVSWFASWGQGTLVTVSS

SEQ ID NO: 18 - protein, 125 aa, synthetic construct
  source 1..125: note = CD3 antibody VH-18
EVQLVESGGGLVQPGGSLRLSCAASGFTFNTYAMNWVRQAPGKGLEWVARIRSKYNNYATYYADSVKDRFTISRDDSKSSLYLQMNSLKTEDTAMYYCVRAGNFGNSYVNWFAYWGQGTLVTVSS

SEQ ID NO: 19 - protein, 125 aa, synthetic construct
  source 1..125: note = CD3 antibody VH-19
EVQLVESGGGLVQPGGSLRLSCAASGFTFNTYAMNWVRQAPGKGLEWVARIRSKYNNYATYYADSVKDRFTISRDDSKSILYLQMNSLKTEDTAVYYCVRHGNFGNSAVSWFQYWGQGTLVTVSS

SEQ ID NO: 20 - protein, 125 aa, synthetic construct
  source 1..125: note = CD3 antibody VH-20
EVQLVESGGGLVQPGGSLRLSCAASGFTFNTYAMNWVRQAPGKGLEWVARIRSKYNNYATYYADSVKDRFTISRDDSKSSLYLQMNSLKTEDTAVYYCVRHGNFGNSYVSWFQYWGQGTLVTVSS

SEQ ID NO: 21 - protein, 125 aa, synthetic construct
  source 1..125: note = CD3 antibody VH-21
EVQLVESGGGLVQPGGSLRLSCAASGFTFNTYAMNWVRQAPGKGLEWVARIRSKYNNYATYYADSVKGRFTISRDDSKSSLYLQMNSLKTEDTAMYYCVRHSNFGNTYVSWFAYWGQGTLVTVSS

SEQ ID NO: 22 - protein, 125 aa, synthetic construct
  source 1..125: note = CD3 antibody VH-22
EVQLVESGGGLVQPGGSLRLSCAASGFTFNTYAMNWVRQAPGKGLEWVARIRSKYNNYATYYADSVKGRFTISRDDSKSILYLQMNSLKTEDTAMYYCVRHERFGNSYVSWFAYWGQGTLVTVSS

SEQ ID NO: 23 - protein, 125 aa, synthetic construct
  source 1..125: note = CD3 antibody VH-23
EVQLVESGGGLVQPGGSLRLSCAASGFTFNTYAMNWVRQAPGKGLEWVARIRSKYNNYATYYADSVKGRFTISRDDSKSILYLQMNSLKTEDTAMYYCVRHSNFLNSYVSWFAYWGQGTLVTVSS

SEQ ID NO: 24 - protein, 125 aa, synthetic construct
  source 1..125: note = CD3 antibody VH-24
EVQLVESGGGLVQPGGSLRLSCAASGFTFNTYAMNWVRQAPGKGLEWVARIRSKYNNYATYYADSVKGRFTISRDDSKSILYLQMNSLKTEDTAVYYCVRHSNFGRSYVSWFAYWGQGTLVTVSS

SEQ ID NO: 25 - protein, 125 aa, synthetic construct
  source 1..125: note = CD3 antibody VH-25
EVQLVESGGGLVQPGGSLRLSCAASGFTFNTYAMNWVRQAPGKGLEWVARIRSKYNNYATYYADSVKDRFTISRDDSKSILYLQMNSLKTEDTAMYYCVRHGNFGNSRVSWFAYWGQGTLVTVSS

SEQ ID NO: 26 - protein, 125 aa, synthetic construct
  source 1..125: note = CD3 antibody VH-26
EVQLVESGGGLVQPGGSLRLSCAASGFTFNTYAMNWVRQAPGKGLEWVARIRSKYNNYATYYADSVKDRFTISRDDSKSILYLQMNNLKTEDTAMYYCVRHGNFGNSQVSWFQYWGQGTLVTVSS

SEQ ID NO: 27 - protein, 125 aa, synthetic construct
  source 1..125: note = CD3 antibody VH-27
EVQLVESGGGLVQPGGSLRLSCAASGFTFNTYAMNWVRQAPGKGLEWVARIRSKYNNYATYYADSVKGRFTISRDDSKSILYLQMNSLKTEDTAMYYCVRHANFGNSYVSWFASWGQGTLVTVSS

SEQ ID NO: 28 - protein, 125 aa, synthetic construct
  source 1..125: note = CD3 antibody VH-28
EVQLVESGGGLVQPGGSLRLSCAASGFTFNTYAMNWVRQAPGKGLEWVARIRSKYNNYATYYADSVKDRFTISRDDSKSILYLQMNSLKTEDTAMYYCVRHHNFGNSYVSWFAYWGQGTLVTVSS

SEQ ID NO: 29 - protein, 125 aa, synthetic construct
  source 1..125: note = CD3 antibody VH-29
EVQLVESGGGLVQPGGSLRLSCAASGFTFNTYAMNWVRQAPGKGLEWVARIRSKYNNYATYYADSVKGRFTISRDDSKSILYLQMNSLKTEDTAMYYCVRHGNFPMSYVSWFAYWGQGTLVTVSS

SEQ ID NO: 30 - protein, 125 aa, synthetic construct
  source 1..125: note = CD3 antibody VH-30
EVQLVESGGGLVQPGGSLRLSCAASGFTFNTYAMNWVRQAPGKGLEWVARIRSKYNNYATYYADSVKDRFTISRDDSKSILYLQMNSLKTEDTAMYYCVRHSNFGNGYVSWFAYWGQGTLVTVSS

SEQ ID NO: 31 - protein, 125 aa, synthetic construct
  source 1..125: note = CD3 antibody VH-31
EVQLVESGGGLVQPGGSLRLSCAASGFTFNTYAMNWVRQAPGKGLEWVARIRSKYNNYATYYADSVKGRFTISRDDSKSILYLQMNNLKTEDTAVYYCVRHSNFGNSYVSWFEYWGQGTLVTVSS

SEQ ID NO: 32 - protein, 125 aa, synthetic construct
  source 1..125: note = CD3 antibody VH-32
EVQLVESGGGLVQPGGSLRLSCAASGFTFNTYAMNWVRQAPGKGLEWVARIRSKYNNYATYYADSVKGRFTISRDDSKSSLYLQMNSLKTEDTAVYYCVRHSNFGNSRVSWFAYWGQGTLVTVSS

SEQ ID NO: 33 - protein, 125 aa, synthetic construct
  source 1..125: note = CD3 antibody VH-33
EVQLVESGGGLVQPGGSLRLSCAASGFTFNTYAMNWVRQAPGKGLEWVARIRSKYNNYATYYADSVKGRFTISRDDSKSSLYLQMNSLKTEDTAVYYCVRHGNFGNNYVSWFASWGQGTLVTVSS

SEQ ID NO: 34 - protein, 125 aa, synthetic construct
  source 1..125: note = CD3 antibody VH-34
EVQLVESGGGLVQPGGSLRLSCAASGFTFNTYAMNWVRQAPGKGLEWVARIRSKYNNYATYYADSVKGRFTISRDDSKSSLYLQMNNLKTEDTAVYYCVRHGNFKQSYVSWFAYWGQGTLVTVSS

SEQ ID NO: 35 - protein, 125 aa, synthetic construct
  source 1..125: note = CD3 antibody VH-35
EVQLVESGGGLVQPGGSLRLSCAASGFTFNTYAMNWVRQAPGKGLEWVARIRSKYNNYATYYADSVKDRFTISRDDSKSSLYLQMNNLKTEDTAVYYCVRHSNFGNSYVSWWAYWGQGTLVTVSS

SEQ ID NO: 36 - protein, 125 aa, synthetic construct
  source 1..125: note = CD3 antibody VH-36
EVQLVESGGGLVQPGGSLRLSCAASGFTFNTYAMNWVRQAPGKGLEWVARIRSKYNNYATYYADSVKDRFTISRDDSKSSLYLQMNSLKTEDTAMYYCVRHSNFPNSYVSWFAYWGQGTLVTVSS

SEQ ID NO: 37 - protein, 125 aa, synthetic construct
  source 1..125: note = CD3 antibody VH-37
EVQLVESGGGLVQPGGSLRLSCAASGFTFNTYAMNWVRQAPGKGLEWVARIRSKYNNYATYYADSVKDRFTISRDDSKSILYLQMNNLKTEDTAMYYCVRHANFSNSYVSWFAYWGQGTLVTVSS

SEQ ID NO: 38 - protein, 125 aa, synthetic construct
  source 1..125: note = CD3 antibody VH-38
EVQLVESGGGLVQPGGSLRLSCAASGFTFNTYAMNWVRQAPGKGLEWVARIRSKYNNYATYYADSVKDRFTISRDDSKSSLYLQMNNLKTEDTAVYYCVRHGNFLNSYVSWFQYWGQGTLVTVSS

SEQ ID NO: 39 - protein, 125 aa, synthetic construct
  source 1..125: note = CD3 antibody VH-39
EVQLVESGGGLVQPGGSLRLSCAASGFTFNTYAMNWVRQAPGKGLEWVARIRSKYNNYATYYADSVKDRFTISRDDSKSSLYLQMNNLKTEDTAMYYCVRHQNFGNSYVSWFQYWGQGTLVTVSS

SEQ ID NO: 40 - protein, 125 aa, synthetic construct
  source 1..125: note = CD3 antibody VH-40
EVQLVESGGGLVQPGGSLRLSCAASGFTFNTYAMNWVRQAPGKGLEWVARIRSKYNNYATYYADSVKDRFTISRDDSKSSLYLQMNNLKTEDTAMYYCVRAGNFGNSYVSWFQYWGQGTLVTVSS

SEQ ID NO: 41 - protein, 125 aa, synthetic construct
  source 1..125: note = CD3 antibody VH-41
EVQLVESGGGLVQPGGSLRLSCAASGFTFNTYAMNWVRQAPGKGLEWVARIRSKYNNYATYYADSVKGRFTISRDDSKSSLYLQMNNLKTEDTAMYYCVRHSNFQNSYVSWFAYWGQGTLVTVSS

SEQ ID NO: 42 - protein, 125 aa, synthetic construct
  source 1..125: note = CD3 antibody VH-42
EVQLVESGGGLVQPGGSLRLSCAASGFTFNTYAMNWVRQAPGKGLEWVARIRSKYNNYATYYADSVKGRFTISRDDSKSSLYLQMNNLKTEDTAMYYCVRHGNFQNSYVSWFQYWGQGTLVTVSS

SEQ ID NO: 43 - protein, 125 aa, synthetic construct
  source 1..125: note = CD3 antibody VH-43
EVQLVESGGGLVQPGGSLRLSCAASGFTFNTYAMNWVRQAPGKGLEWVARIRSKYNNYATYYADSVKDRFTISRDDSKSILYLQMNSLKTEDTAMYYCVRPGNFPNSYVSWFALWGQGTLVTVSS

SEQ ID NO: 44 - protein, 125 aa, synthetic construct
  source 1..125: note = CD3 antibody VH-44
EVQLVESGGGLVQPGGSLRLSCAASGFTFNTYAMNWVRQAPGKGLEWVARIRSKYNNYATYYADSVKDRFTISRDDSKSSLYLQMNNLKTEDTAMYYCVRHGNFQNSYISWFAYWGQGTLVTVSS

SEQ ID NO: 45 - protein, 125 aa, synthetic construct
  source 1..125: note = CD3 antibody VH-45
EVQLVESGGGLVQPGGSLRLSCAASGFTFNTYAMNWVRQAPGKGLEWVARIRSKYNNYATYYADSVKDRFTISRDDSKSSLYLQMNNLKTEDTAMYYCVRHSNFGNSYVSWFQYWGQGTLVTVSS

SEQ ID NO: 46 - protein, 125 aa, synthetic construct
  source 1..125: note = CD3 antibody VH-46
EVQLVESGGGLVQPGGSLRLSCAASGFTFNTYAMNWVRQAPGKGLEWVARIRSKYNNYATYYADSVKDRFTISRDDSKSILYLQMNSLKTEDTAMYYCVRHANFGNSYVSWFASWGQGTLVTVSS

SEQ ID NO: 47 - protein, 109 aa, synthetic construct
  source 1..109: note = CD3 antibody VL-1
QAVVTQEPSFSVSPGGTVTLTCRSSTGAVTTSNYANWVQQTPGQAFRGLIGGTNKRAPGVPARFSGSLIGDKAALTITGAQADDESIYFCALWYSNLWVFGGGTKLTVL

SEQ ID NO: 48 - protein, 109 aa, synthetic construct
  source 1..109: note = CD3 antibody VL-2
QAVVTQEPSFSVSPGGTVTLTCRSSTGAVTTSNYANWYQQTPGQAPRTLIYGTNKRAPGVPARFSGSILGNKAALTITGAQADDESDYFCALWYSNLWVFGGGTKLTVL

SEQ ID NO: 49 - protein, 14 aa, synthetic construct
  source 1..14: note = HCDR3 (VH1)
HANFLNSYVSWFAY

SEQ ID NO: 50 - protein, 14 aa, synthetic construct
  source 1..14: note = HCDR3 (VH2)
AKNFGNSYVSWFAY

SEQ ID NO: 51 - protein, 14 aa, synthetic construct
  source 1..14: note = HCDR3 (VH3)
HGNFGNSYVSWFEY

SEQ ID NO: 52 - protein, 14 aa, synthetic construct
  source 1..14: note = HCDR3 (VH4/VH42)
HGNFQNSYVSWFQY

SEQ ID NO: 53 - protein, 14 aa, synthetic construct
  source 1..14: note = HCDR3 (VH5)
HGNFKNSYVSWFAY

SEQ ID NO: 54 - protein, 14 aa, synthetic construct
  source 1..14: note = HCDR3 (VH6)
HGNFYNSYVSWFAH

SEQ ID NO: 55 - protein, 14 aa, synthetic construct
  source 1..14: note = HCDR3 (VH7)
AGNFGNSYVSWFEY

SEQ ID NO: 56 - protein, 14 aa, synthetic construct
  source 1..14: note = HCDR3 (VH8)
HGNFGNTYVSWFAM

SEQ ID NO: 57 - protein, 14 aa, synthetic construct
  source 1..14: note = HCDR3 (VH9)
HGNFGNSYVSWFKY

SEQ ID NO: 58 - protein, 14 aa, synthetic construct
  source 1..14: note = HCDR3 (VH10)
HSNFRNSYVSWFAY

SEQ ID NO: 59 - protein, 14 aa, synthetic construct
  source 1..14: note = HCDR3 (VH11)
HSNFVNSYVSWFAY

SEQ ID NO: 60 - protein, 14 aa, synthetic construct
  source 1..14: note = HCDR3 (VH12/VH36)
HSNFPNSYVSWFAY

SEQ ID NO: 61 - protein, 14 aa, synthetic construct
  source 1..14: note = HCDR3 (VH13)
HGNFKNSYGSWFAY

SEQ ID NO: 62 - protein, 14 aa, synthetic construct
  source 1..14: note = HCDR3 (VH14/VH31)
HSNFGNSYVSWFEY

SEQ ID NO: 63 - protein, 14 aa, synthetic construct
  source 1..14: note = HCDR3 (VH15)
HGDPGNSYVSWFAY

SEQ ID NO: 64 - protein, 14 aa, synthetic construct
  source 1..14: note = HCDR3 (VH16/VH20)
HGNFGNSYVSWFQY

SEQ ID NO: 65 - protein, 14 aa, synthetic construct
  source 1..14: note = HCDR3 (VH17)
HGNFWNSYVSWFAS

SEQ ID NO: 66 - protein, 14 aa, synthetic construct
  source 1..14: note = HCDR3 (VH18)
AGNFGNSYVNWFAY

SEQ ID NO: 67 - protein, 14 aa, synthetic construct
  source 1..14: note = HCDR3 (VH19)
HGNFGNSAVSWFQY

SEQ ID NO: 68 - protein, 14 aa, synthetic construct
  source 1..14: note = HCDR3 (VH21)
HSNFGNTYVSWFAY

SEQ ID NO: 69 - protein, 14 aa, synthetic construct
  source 1..14: note = HCDR3 (VH22)
HERFGNSYVSWFAY

SEQ ID NO: 70 - protein, 14 aa, synthetic construct
  source 1..14: note = HCDR3 (VH23)
HSNFLNSYVSWFAY

SEQ ID NO: 71 - protein, 14 aa, synthetic construct
  source 1..14: note = HCDR3 (VH24)
HSNFGRSYVSWFAY

SEQ ID NO: 72 - protein, 14 aa, synthetic construct
  source 1..14: note = HCDR3 (VH25)
HGNFGNSRVSWFAY

SEQ ID NO: 73 - protein, 14 aa, synthetic construct
  source 1..14: note = HCDR3 (VH26)
HGNFGNSQVSWFQY

SEQ ID NO: 74 - protein, 14 aa, synthetic construct
  source 1..14: note = HCDR3 (VH27/VH46)
HANFGNSYVSWFAS

SEQ ID NO: 75 - protein, 14 aa, synthetic construct
  source 1..14: note = HCDR3 (VH28)
HHNFGNSYVSWFAY

SEQ ID NO: 76 - protein, 14 aa, synthetic construct
  source 1..14: note = HCDR3 (VH29)
HGNFPMSYVSWFAY

SEQ ID NO: 77 - protein, 14 aa, synthetic construct
  source 1..14: note = HCDR3 (VH30)
HSNFGNGYVSWFAY

SEQ ID NO: 78 - protein, 14 aa, synthetic construct
  source 1..14: note = HCDR3 (VH32)
HSNFGNSRVSWFAY

SEQ ID NO: 79 - protein, 14 aa, synthetic construct
  source 1..14: note = HCDR3 (VH33)
HGNFGNNYVSWFAS

SEQ ID NO: 80 - protein, 14 aa, synthetic construct
  source 1..14: note = HCDR3 (VH34)
HGNFKQSYVSWFAY

SEQ ID NO: 81 - protein, 14 aa, synthetic construct
  source 1..14: note = HCDR3 (VH35)
HSNFGNSYVSWWAY

SEQ ID NO: 82 - protein, 14 aa, synthetic construct
  source 1..14: note = HCDR3 (VH37)
HANFSNSYVSWFAY

SEQ ID NO: 83 - protein, 14 aa, synthetic construct
  source 1..14: note = HCDR3 (VH38)
HGNFLNSYVSWFQY

SEQ ID NO: 84 - protein, 14 aa, synthetic construct
  source 1..14: note = HCDR3 (VH39)
HQNFGNSYVSWFQY

SEQ ID NO: 85 - protein, 14 aa, synthetic construct
  source 1..14: note = HCDR3 (VH40)
AGNFGNSYVSWFQY

SEQ ID NO: 86 - protein, 14 aa, synthetic construct
  source 1..14: note = HCDR3 (VH41)
HSNFQNSYVSWFAY

SEQ ID NO: 87 - protein, 14 aa, synthetic construct
  source 1..14: note = HCDR3 (VH43)
PGNFPNSYVSWFAL

SEQ ID NO: 88 - protein, 14 aa, synthetic construct
  source 1..14: note = HCDR3 (VH44)
HGNFQNSYISWFAY

SEQ ID NO: 89 - protein, 14 aa, synthetic construct
  source 1..14: note = HCDR3 (VH45)
HSNFGNSYVSWFQY

SEQ ID NO: 90 - protein, 14 aa, synthetic construct
  source 1..14: note = HCDR3
HGNFGNSYVSWFAY

SEQ ID NO: 91 - protein, 35 aa, synthetic construct
  source 1..35: note = HFR3 (VH1)
VKGRFTISRDDSKSILYLQMNNLKTEDTAMYYCVR

SEQ ID NO: 92 - protein, 35 aa, synthetic construct
  source 1..35: note = HFR3 (VH2/VH6/VH21)
VKGRFTISRDDSKSSLYLQMNSLKTEDTAMYYCVR

SEQ ID NO: 93 - protein, 35 aa, synthetic construct
  source 1..35: note = HFR3 (VH3/VH17/VH25/VH28/VH30/VH43/VH46)
VKDRFTISRDDSKSILYLQMNSLKTEDTAMYYCVR

SEQ ID NO: 94 - protein, 35 aa, synthetic construct
  source 1..35: note = HFR3 (VH4)
VKDRFTISRDDSKSILYLQMNNLKTEDTAVYYCVR

SEQ ID NO: 95 - protein, 35 aa, synthetic construct
  source 1..35: note = HFR3 (VH5/VH19)
VKDRFTISRDDSKSILYLQMNSLKTEDTAVYYCVR

SEQ ID NO: 96 - protein, 35 aa, synthetic construct
  source 1..35: note = HFR3 (VH7/VH8/VH39/VH40/VH44/VH45)
VKDRFTISRDDSKSSLYLQMNNLKTEDTAMYYCVR

SEQ ID NO: 97 - protein, 35 aa, synthetic construct
  source 1..35: note = HFR3 (VH9/VH22/VH23/VH27/VH29)
VKGRFTISRDDSKSILYLQMNSLKTEDTAMYYCVR

SEQ ID NO: 98 - protein, 35 aa, synthetic construct
  source 1..35: note = HFR3 (VH10/VH11/VH20)
VKDRFTISRDDSKSSLYLQMNSLKTEDTAVYYCVR

SEQ ID NO: 99 - protein, 35 aa, synthetic construct
  source 1..35: note = HFR3 (VH12/VH41/VH42)
VKGRFTISRDDSKSSLYLQMNNLKTEDTAMYYCVR

SEQ ID NO: 100 - protein, 35 aa, synthetic construct
  source 1..35: note = HFR3 (VH13/VH32/VH33)
VKGRFTISRDDSKSSLYLQMNSLKTEDTAVYYCVR

SEQ ID NO: 101 - protein, 35 aa, synthetic construct
  source 1..35: note = HFR3 (VH14/VH15/VH18/VH36)
VKDRFTISRDDSKSSLYLQMNSLKTEDTAMYYCVR

SEQ ID NO: 102 - protein, 35 aa, synthetic construct
  source 1..35: note = HFR3 (VH16/VH24)
VKGRFTISRDDSKSILYLQMNSLKTEDTAVYYCVR

SEQ ID NO: 103 - protein, 35 aa, synthetic construct
  source 1..35: note = HFR3 (VH26/VH37)
VKDRFTISRDDSKSILYLQMNNLKTEDTAMYYCVR

SEQ ID NO: 104 - protein, 35 aa, synthetic construct
  source 1..35: note = HFR3 (VH31)
VKGRFTISRDDSKSILYLQMNNLKTEDTAVYYCVR

SEQ ID NO: 105 - protein, 35 aa, synthetic construct
  source 1..35: note = HFR3 (VH34)
VKGRFTISRDDSKSSLYLQMNNLKTEDTAVYYCVR

SEQ ID NO: 106 - protein, 35 aa, synthetic construct
  source 1..35: note = HFR3 (VH35/VH38)
VKDRFTISRDDSKSSLYLQMNNLKTEDTAVYYCVR

SEQ ID NO: 107 - protein, 5 aa, synthetic construct
  source 1..5: note = HCDR1
TYAMN

SEQ ID NO: 108 - protein, 15 aa, synthetic construct
  source 1..15: note = HCDR2
IRSKYNNYATYYADS

SEQ ID NO: 109 - protein, 30 aa, synthetic construct
  source 1..30: note = HFR1
EVQLVESGGGLVQPGGSLRLSCAASGFTFN

SEQ ID NO: 110 - protein, 15 aa, synthetic construct
  source 1..15: note = HFR2
WVRQAPGKGLEWVAR

SEQ ID NO: 111 - protein, 11 aa, synthetic construct
  source 1..11: note = HFR4
WGQGTLVTVSS

SEQ ID NO: 112 - skipped

SEQ ID NO: 113 - protein, 14 aa, synthetic construct
  source 1..14: note = HCDR3 general formula
  VARIANT 2: note = X is A, E, H, K, Q or S
HXNFGNSYVSWFAY

SEQ ID NO: 114 - protein, 14 aa, synthetic construct
  source 1..14: note = HCDR3 general formula
  VARIANT 5: note = X is K, L, P, Q, R, S, V, W or Y
HGNFXNSYVSWFAY

SEQ ID NO: 115 - protein, 14 aa, synthetic construct
  source 1..14: note = HCDR3 general formula
  VARIANT 8: note = X is A, Q or R
HGNFGNSXVSWFAY

SEQ ID NO: 116 - protein, 14 aa, synthetic construct
  source 1..14: note = HCDR3 general formula
  VARIANT 13: note = X is E, K or Q
HGNFGNSYVSWFXY

SEQ ID NO: 117 - protein, 14 aa, synthetic construct
  source 1..14: note = HCDR3 general formula
  VARIANT 1: note = X is A or P
  VARIANT 2: note = X is A, E, H, K, Q or S
XXNFGNSYVSWFAY

SEQ ID NO: 118 - protein, 14 aa, synthetic construct
  source 1..14: note = HCDR3 general formula
  VARIANT 1: note = X1 is A or P
  VARIANT 10: note = X is N
XGNFGNSYVXWFAY

SEQ ID NO: 119 - protein, 14 aa, synthetic construct
  source 1..14: note = HCDR3 general formula
  VARIANT 1: note = X is A or P
  VARIANT 13: note = X is E, K or Q
XGNFGNSYVSWFXY

SEQ ID NO: 120 - protein, 14 aa, synthetic construct
  source 1..14: note = HCDR3 general formula
  VARIANT 2: note = X is A, E, H, K, Q or S
  VARIANT 3: note = X is D or R
HXXFGNSYVSWFAY

SEQ ID NO: 121 - protein, 14 aa, synthetic construct
  source 1..14: note = HCDR3 general formula
  VARIANT 2: note = X is A, E, H, K, Q or S
  VARIANT 5: note = X is K, L, P, Q, R, S, V, W or Y
HXNFXNSYVSWFAY

SEQ ID NO: 122 - protein, 14 aa, synthetic construct
  source 1..14: note = HCDR3 general formula
  VARIANT 2: note = X is A, E, H, K, Q or S
  VARIANT 6: note = X is M, Q or R
HXNFGXSYVSWFAY

SEQ ID NO: 123 - protein, 14 aa, synthetic construct
  source 1..14: note = HCDR3 general formula
  VARIANT 2: note = X is A, E, H, K, Q or S
  VARIANT 7: note = X is G, N or T
HXNFGNXYVSWFAY

SEQ ID NO: 124 - protein, 14 aa, synthetic construct
  source 1..14: note = HCDR3 general formula
  VARIANT 2: note = X is A, E, H, K, Q or S
  VARIANT 8: note = X is A, Q or R
HXNFGNSXVSWFAY

SEQ ID NO: 125 - protein, 14 aa, synthetic construct
  source 1..14: note = HCDR3 general formula
  VARIANT 2: note = X is A, E, H, K, Q or S
  VARIANT 12: note = X is W
HXNFGNSYVSWXAY

SEQ ID NO: 126 - protein, 14 aa, synthetic construct
  source 1..14: note = HCDR3 general formula
  VARIANT 2: note = X is A, E, H, K, Q or S
  VARIANT 13: note = X is E, K or Q
HXNFGNSYVSWFXY

SEQ ID NO: 127 - protein, 14 aa, synthetic construct
  source 1..14: note = HCDR3 general formula
  VARIANT 2: note = X is A, E, H, K, Q or S
  VARIANT 14: note = X is H, L, M or S
HXNFGNSYVSWFAX

SEQ ID NO: 128 - protein, 14 aa, synthetic construct
  source 1..14: note = HCDR3 general formula
  VARIANT 3: note = X is D or R
  VARIANT 4: note = X is P
HGXXGNSYVSWFAY

SEQ ID NO: 129 - protein, 14 aa, synthetic construct
  source 1..14: note = HCDR3 general formula
  VARIANT 5: note = X is K, L, P, Q, R, S, V, W or Y
  VARIANT 6: note = X is M, Q or R
HGNFXXSYVSWFAY

SEQ ID NO: 130 - protein, 14 aa, synthetic construct
  source 1..14: note = HCDR3 general formula
  VARIANT 5: note = X is K, L, P, Q, R, S, V, W or Y
  VARIANT 9: note = X is G or I
HGNFXNSYXSWFAY

SEQ ID NO: 131 - protein, 14 aa, synthetic construct
  source 1..14: note = HCDR3 general formula
  VARIANT 5: note = X is K, L, P, Q, R, S, V, W or Y
  VARIANT 13: note = X is E, K or Q
HGNFXNSYVSWFXY

SEQ ID NO: 132 - protein, 14 aa, synthetic construct
  source 1..14: note = HCDR3 general formula
  VARIANT 5: note = X is K, L, P, Q, R, S, V, W or Y
  VARIANT 14: note = X is H, L, M or S
HGNFXNSYVSWFAX

SEQ ID NO: 133 - protein, 14 aa, synthetic construct
  source 1..14: note = HCDR3 general formula
  VARIANT 7: note = X is G, N or T
  VARIANT 14: note = X is H, L, M or S
HGNFGNXYVSWFAX

SEQ ID NO: 134 - protein, 14 aa, synthetic construct
  source 1..14: note = HCDR3 general formula
  VARIANT 8: note = X is A, Q or R
  VARIANT 13: note = X is E, K or Q
HGNFGNSXVSWFXY

SEQ ID NO: 135 - protein, 14 aa, synthetic construct
  source 1..14: note = HCDR3 general formula
  VARIANT 1: note = X is A or P
  VARIANT 5: note = X is K, L, P, Q, R, S, V, W or Y
  VARIANT 14: note = X is H, L, M or S
XGNFXNSYVSWFAX

SEQ ID NO: 136 - protein, 35 aa, synthetic construct
  source 1..35: note = HFR3 general formula
  VARIANT 3: note = X is G or D
  VARIANT 15: note = X is I or S
  VARIANT 22: note = X is N or S
  VARIANT 30: note = X is M or V
VKXRFTISRDDSKSXLYLQMNXLKTEDTAXYYCVR

SEQ ID NO: 137 - protein, 13 aa, synthetic construct
  source 1..13: note = LCDR1 (VL1/VL2)
SSTGAVTTSNYAN

SEQ ID NO: 138 - protein, 7 aa, synthetic construct
  source 1..7: note = LCDR2 (VL1/VL2)
GTNKRAP

SEQ ID NO: 139 - protein, 8 aa, synthetic construct
  source 1..8: note = LCDR3 (VL1/VL2)
LWYSNLWV

SEQ ID NO: 140 - protein, 23 aa, synthetic construct
  source 1..23: note = LFR1 (VL1/VL2)
QAVVTQEPSFSVSPGGTVTLTCR

SEQ ID NO: 141 - protein, 10 aa, synthetic construct
  source 1..10: note = LFR4 (VL1/VL2)
FGGGTKLTVL

SEQ ID NO: 142 - protein, 15 aa, synthetic construct
  source 1..15: note = LFR2 (VL1)
WVQQTPGQAFRGLIG

SEQ ID NO: 143 - protein, 15 aa, synthetic construct
  source 1..15: note = LFR2 (VL2)
WYQQTPGQAPRTLIY

SEQ ID NO: 144 - protein, 15 aa, synthetic construct
  source 1..15: note = LFR2 general formula
  VARIANT 2: note = X is V or Y
  VARIANT 10: note = X is F or P
  VARIANT 12: note = X is G or T
  VARIANT 15: note = X is G or Y
WXQQTPGQAXRXLIX

SEQ ID NO: 145 - protein, 33 aa, synthetic construct
  source 1..33: note = LFR3 (VL1)
GVPARFSGSLIGDKAALTITGAQADDESIYFCA

SEQ ID NO: 146 - protein, 33 aa, synthetic construct
  source 1..33: note = LFR3 (VL2)
GVPARFSGSILGNKAALTITGAQADDESDYFCA

SEQ ID NO: 147 - protein, 33 aa, synthetic construct
  source 1..33: note = LFR3 general formula
  VARIANT 10: note = X is L or I
  VARIANT 11: note = X is L or I
  VARIANT 13: note = X is D or N
  VARIANT 29: note = X is I or D
GVPARFSGSXXGXKAALTITGAQADDESXYFCA

SEQ ID NO: 148 - protein, 14 aa, synthetic construct
  source 1..14: note = HCDR3 general formula
  VARIANT 1: note = X is H or P
  VARIANT 2: note = X is G, E, or A
  VARIANT 3: note = X is N or R
  VARIANT 5: note = X is G, K, S, or P
  VARIANT 7: note = X is T, S, or N
  VARIANT 9: note = X is V or G
  VARIANT 14: note = X is M, Y, S, or L
XXXFXNXYXSWFAX

SEQ ID NO: 149 - protein, 115 aa, synthetic construct
  source 1..115: note = MSLN VHH
EVQLVESGGGLVQAGESLRLSCAVSGNIGSIRHMGWHRQDPGKERELVATITTVGTTYYANFVKGRFTISRDNAKNTVYLQMNSLKPEDTGVYYCRATAHPTDYWGQGTQVTVSS

SEQ ID NO: 150 - protein, 8 aa, synthetic construct
  source 1..8: note = MSLN VHH-CDR1(IMGT)
GNIGSIRH

SEQ ID NO: 151 - protein, 7 aa, synthetic construct
  source 1..7: note = MSLN VHH-CDR2(IMGT)
ITTVGTT

SEQ ID NO: 152 - protein, 9 aa, synthetic construct
  source 1..9: note = MSLN VHH-CDR3(IMGT)
RATAHPTDY

SEQ ID NO: 153 - protein, 5 aa, synthetic construct
  source 1..5: note = MSLN VHH-CDR1(Kabat)
IRHMG

SEQ ID NO: 154 - protein, 16 aa, synthetic construct
  source 1..16: note = MSLN VHH-CDR2(Kabat)
TITTVGTTYYANFVKG

SEQ ID NO: 155 - protein, 7 aa, synthetic construct
  source 1..7: note = MSLN VHH-CDR3(Kabat/ AbM/ Chothia)
TAHPTDY

SEQ ID NO: 156 - protein, 10 aa, synthetic construct
  source 1..10: note = MSLN VHH-CDR1(AbM)
GNIGSIRHMG

SEQ ID NO: 157 - protein, 9 aa, synthetic construct
  source 1..9: note = MSLN VHH-CDR2(AbM)
TITTVGTTY

SEQ ID NO: 158 - protein, 7 aa, synthetic construct
  source 1..7: note = MSLN VHH-CDR1(Chothia)
GNIGSIR

SEQ ID NO: 159 - protein, 5 aa, synthetic construct
  source 1..5: note = MSLN VHH-CDR2(Chothia)
TTVGT

SEQ ID NO: 160 - protein, 6 aa, synthetic construct
  source 1..6: note = MSLN VHH-CDR1(Contact)
SIRHMG

SEQ ID NO: 161 - protein, 12 aa, synthetic construct
  source 1..12: note = MSLN VHH-CDR2(Contact)
LVATITTVGTTY

SEQ ID NO: 162 - protein, 8 aa, synthetic construct
  source 1..8: note = MSLN VHH-CDR3(Contact)
RATAHPTD

SEQ ID NO: 163 - protein, 10 aa, synthetic construct
  source 1..10: note = Linker
GGGGSGGGGS

SEQ ID NO: 164 - protein, 329 aa, synthetic construct
  source 1..329: note = IgG1 heavy chain constant region
ASTKGPSVFPLAPSSKSTSGGTAALGCLVKDYFPEPVTVSWNSGALTSGVHTFPAVLQSSGLYSLSSVVTVPSSSLGTQTYICNVNHKPSNTKVDKKVEPKSCDKTHTCPPCPAPEAAGAPSVFLFPPKPKDTLMISRTPEVTCVVVDVSHEDPEVKFNWYVDGVEVHNAKTKPREEQYNSTYRVVSVLTVLHQDWLNGKEYKCAVSNKALPAPIEKTISKAKGQPREPQVYTLPPSRDELTKNQVSLTCLVKGFYPSDIAVEWESNGQPENNYKTTPPVLDSDGSFFLYSKLTVDKSRWQQGNVFSCSVMHEALHNHYTQKSLSLSPG

SEQ ID NO: 165 - protein, 106 aa, synthetic construct
  source 1..106: note = Light chain constant region
GQPKAAPSVTLFPPSSEELQANKATLVCLISDFYPGAVTVAWKADSSPVKAGVETTTPSKQSNNKYAASSYLSLTPEQWKSHRSYSCQVTHEGSTVEKTVAPTECS

SEQ ID NO: 166 - protein, 119 aa, synthetic construct [sequence omitted]

SEQ ID NO: 167 - protein, 105 aa, synthetic construct
  source 1..105: note = Positive control antibody OKT3-VL
QIVLTQSPAIMSASPGEKVTMTCSASSSVSYMNWYQQKSGTSPKRWIYDTSKLASGVPAHFRGSGSGTSYSLTISGMEAEDAATYYCQQWSSNPFTFGSGTKLEI

SEQ ID NO: 168 - protein, 125 aa, synthetic construct
  source 1..125: note = Control antibody 1-VH
EVQLVESGGGLVQPKGSLKLSCAASGFTFNTYAMNWVRQAPGKGLEWVARIRSKYNNYATYYADSVKDRFTISRDDSQSILYLQMNNLKTEDTAMYYCVRHGNFGNSYVSWFAYWGQGTLVTVSA

SEQ ID NO: 169 - protein, 109 aa, synthetic construct
  source 1..109: note = Control antibody 1-VL
QAVVTQESALTTSPGETVTLTCRSSTGAVTTSNYANWVQEKPDHLFTGLIGGTNKRAPGVPARFSGSLIGDKAALTITGAQTEDEAIYFCALWYSNLWVFGGGTKLTVL

SEQ ID NO: 170 - protein, 124 aa, synthetic construct
  source 1..124: note = Anti-CD19 VH
QVQLQQSGAELVRPGSSVKISCKASGYAFSSYWMNWVKQRPGQGLEWIGQIWPGDGDTNYNGKFKGKATLTADESSSTAYMQLSSLASEDSAVYFCARRETTTVGRYYYAMDYWGQGTTVTVSS

SEQ ID NO: 171 - protein, 111 aa, synthetic construct
  source 1..111: note = Anti-CD19 VL
DIQLTQSPASLAVSLGQRATISCKASQSVDYDGDSYLNWYQQIPGQPPKLLIYDASNLVSGIPPRFSGSGSGTDFTLNIHPVEKVDAATYHCQQSTEDPWTFGGGTKLEIK

SEQ ID NO: 172 - protein, 119 aa, synthetic construct
  source 1..119: note = Anti-CD20 VH
QVQLVQSGAEVKKPGSSVKVSCKASGYAFSYSWINWVRQAPGQGLEWMGRIFPGDGDTDYNGKFKGRVTITADKSTSTAYMELSSLRSEDTAVYYCARNVFDGYWLVYWGQGTLVTVSS

SEQ ID NO: 173 - protein, 112 aa, synthetic construct
  source 1..112: note = Anti-CD20 VL
DIVMTQTPLSLPVTPGEPASISCRSSKSLLHSNGITYLYWYLQKPGQSPQLLIYQMSNLVSGVPDRFSGSGSGTDFTLKISRVEAEDVGVYYCAQNLELPYTFGGGTKVEIK

SEQ ID NO: 174 - protein, 128 aa, synthetic construct
  source 1..128: note = Anti-trop2 VHH
EVQLVESGGGLVQPGGSLRLSCAASGFTLGDYAIGWFRQAPGKEREGVSCISSTGGVTNYADSVKGRFTISRDNAKNTVYLQMNSLKPEDTAVYYCAANYYSDYDCPPAFYSYVMDYWGKGTLVTVSS

SEQ ID NO: 175 - protein, 124 aa, synthetic construct
  source 1..124: note = Anti-Her2 VHH
EVQLVESGGSLVQPGGSLRLSCAASGFTFDDYAMSWVRQVPGKGLEWVSSINWSGTHTDYADSVKGRFTISRNNANNTLYLQMNSLKSEDTAVYYCAKNWRDAGTTWFEKSGSAGQGTQVTVSS

SEQ ID NO: 176 - protein, 116 aa, synthetic construct
  source 1..116: note = Anti-Caludin18.2 VHH
QVQLVESGGGLVQAGGSLKLSCTASGDRFSSYAMGWFRQAPGKEREFVAAVSWSGRITDYADSVKGRFTISRDNAKDTVYLQMNNLKPEDTSVYYCYANLLWRDHWGQGTLVTVSS